European Patent Application EP 4 421 090 A1, published August 28, 2024. Title: FC VARIANTS HAVING IMPROVED PH-DEPENDENT FCRN BINDING CAPACITY AND FCΓRⅢA BINDING SELECTIVITY. Applicant: KOREA UNIVERSITY RESEARCH AND BUSINESS FOUNDATION. The sequence listing filed with the application follows.

SEQUENCE LISTING (10 sequences)

SEQ ID NO: 1 - protein, 227 aa, synthetic construct
DKTHTCPPCPAPELPGGPSVFLFPPKPKDTLMISRTPEITCVVVDVSHEDPEVKFNWYVDGVEVHNAKTKPREEQYNSTYRVVSVLTVLHRDWLNGKEYKCKVSNKALPAPEEKTISKAKGQPREPQVYTLPPSRDELTKNQVSLTCLVKGFYPSDIVVEWESNGQPENNYKTTPPVLDSDGSFFLYSKLTVDKSRWQQGNVFSCSVLHEALHNHYTQKSLSLSPGK

SEQ ID NO: 2 - DNA, 681 bp, synthetic construct
  source 1..681: mol_type = other DNA
gacaaaactcacacatgcccaccgtgcccagcacctgaactcccggggggaccgtcagtcttcctcttccccccaaaacccaaggacaccctcatgatctcccggacccctgagatcacatgcgtggtggtggacgtgagccacgaagaccctgaggtcaagttcaactggtacgtggacggcgtggaggtgcataatgccaagacaaagccgcgggaggagcagtacaacagcacgtaccgtgtggtcagcgtcctcaccgtcctgcaccgtgactggctgaatggcaaggagtacaagtgcaaggtctccaacaaagccctcccagcccccgaggagaaaaccatctccaaagccaaagggcagccccgagaaccacaggtgtacaccctgcccccatcccgggatgagctgaccaagaaccaggtcagcctgacctgcctggtcaaaggcttctatcccagcgacatcgtcgtggagtgggagagcaatgggcagccggagaacaactacaagaccacacctcccgtgctggactccgacggctccttcttcctctacagcaagctcaccgtggacaagagcaggtggcagcaggggaacgtcttctcatgctccgtgctgcatgaggctctgcacaaccactacacgcagaagagcctctccctgtctccgggtaaa

SEQ ID NO: 3 - protein, 227 aa, synthetic construct
DKTHTCPPCPAPELLGGPDVFLFPPKPKDTLMISRTPEVTCVVVDVSLEDPEVKFNWYVDGVEVHNAKTKPREEQYNSTYRVVSVLTVLHRDWLNGKEYKCKVSNKALPVPEEKTISKAKGQPREPQVYTLPPSRDELTKNQVSLTCLVKGFYPSDIAVEWESNGQPENNYKTTPPVLDSDGSFFLYSKLTVDKSRWQQGNVFSCSVLHEALHNHYTQKSLSLSPGK

SEQ ID NO: 4 - DNA, 681 bp, synthetic construct
  source 1..681: mol_type = other DNA
gacaaaactcacacatgcccaccgtgcccagcacctgaactcctggggggaccggacgtcttcctcttccccccaaaacccaaggacaccctcatgatctcccggacccctgaggtcacatgcgtggtggtggacgtgagcctcgaagaccctgaggtcaagttcaactggtacgtggacggcgtggaggtgcataatgccaagacaaagccgcgggaggagcagtacaacagcacgtaccgtgtggtcagcgtcctcaccgtcctgcaccgtgactggctgaatggcaaggagtacaagtgcaaggtctccaacaaagccctcccagtccccgaggagaaaaccatctccaaagccaaagggcagccccgagaaccacaggtgtacaccctgcccccatcccgggatgagctgaccaagaaccaggtcagcctgacctgcctggtcaaaggcttctatcccagcgacatcgccgtggagtgggagagcaatgggcagccggagaacaactacaagaccacacctcccgtgctggactccgacggctccttcttcctctacagcaagctcaccgtggacaagagcaggtggcagcaggggaacgtcttctcatgctccgtgctgcatgaggctctgcacaaccactacacgcagaagagcctctccctgtctccgggtaaa

SEQ ID NO: 5 - protein, 227 aa, synthetic construct
DKTHTCPPCPAPELLGGPDVFLFPPKPMDTLMISRTPEVTCVVVDVSLEDPEVKFNWYVDGVEVHNAKTKPREEQYNSTYRVVSVLTVEHMDWLNGKEYKCKVSNKALPVPEEKTISKAKGQPREPQVYTLPPSRDELTKNQVSLTCLVKGFYPSDIAVEWESNGQPENNYKTTPPVLDSDGSFFLYSKLTVDKSRWQQGNVFSCSVLHEALHNHYTQKSLSLSPGK

SEQ ID NO: 6 - DNA, 681 bp, synthetic construct
  source 1..681: mol_type = other DNA
gacaaaactcacacatgcccaccgtgcccagcacctgaactcctggggggaccggacgtcttcctcttccccccaaaacccatggacaccctcatgatctcccggacccctgaggtcacatgcgtggtggtggacgtgagcctcgaagaccctgaggtcaagttcaactggtacgtggacggcgtggaggtgcataatgccaagacaaagccgcgggaggagcagtacaacagcacgtaccgtgtggtcagcgtcctcaccgtcgaacacatggactggctgaatggcaaggagtacaagtgcaaggtctccaacaaagccctcccagtccccgaggagaaaaccatctccaaagccaaagggcagccccgagaaccacaggtgtacaccctgcccccatcccgggatgagctgaccaagaaccaggtcagcctgacctgcctggtcaaaggcttctatcccagcgacatcgccgtggagtgggagagcaatgggcagccggagaacaactacaagaccacacctcccgtgctggactccgacggctccttcttcctctacagcaagctcaccgtggacaagagcaggtggcagcaggggaacgtcttctcatgctccgtgctgcatgaggctctgcacaaccactacacgcagaagagcctctccctgtctccgggtaaa

SEQ ID NO: 7 - protein, 227 aa, synthetic construct
DKTHTCPPCPAPELPGGPDVFLFPPKPKDTLMISRTPEVTCVVVDVSHEYPEVKFNWYVDGVEVHNAKTKPREEQYNGTYRVVSVLTVLHRDWLNGKEYKCKVSNKALPAPEEKTISKAKGQPREPQVYTLPPSRGELTKNQVSLTCLVKGFYPSDIAVEWESNGQPENNYKTTPPVLDSDGSFFLYSKLTVDKSRWQQGNVFSCSVLHEALHNHYTQKSLSLSPGK

SEQ ID NO: 8 - DNA, 681 bp, synthetic construct
  source 1..681: mol_type = other DNA
gacaaaactcacacatgcccaccgtgcccagcacctgaactcccggggggaccggacgtcttcctcttccccccaaaacccaaggacaccctcatgatctcccggacccctgaggtcacatgcgtggtggtggacgtgagccacgaataccctgaggtcaagttcaactggtacgtggacggcgtggaggtgcataatgccaagacaaagccgcgggaggagcagtacaacggcacgtaccgtgtggtcagcgtcctcaccgtcctgcaccgtgactggctgaatggcaaggagtacaagtgcaaggtctccaacaaagccctcccagcccccgaggagaaaaccatctccaaagccaaagggcagccccgagaaccacaggtgtacaccctgcccccatcccggggtgagctgaccaagaaccaggtcagcctgacctgcctggtcaaaggcttctatcccagcgacatcgccgtggagtgggagagcaatgggcagccggagaacaactacaagaccacacctcccgtgctggactccgacggctccttcttcctctacagcaagctcaccgtggacaagagcaggtggcagcaggggaacgtcttctcatgctccgtgctgcatgaggctctgcacaaccactacacgcagaagagcctctccctgtccccgggtaaa

SEQ ID NO: 9 - protein, 227 aa, synthetic construct
DKTHTCPPCPAPELLGGPSVFLFPPKPKDTLMISRTPEVTCVVVDVSHEDPEVKFNWYVDGVEVHNAKTKPREEQYNSTYRVVSVLTVLHQDWLNGKEYKCKVSNKALPAPIEKTISKAKGQPREPQVYTLPPSRDELTKNQVSLTCLVKGFYPSDIAVEWESNGQPENNYKTTPPVLDSDGSFFLYSKLTVDKSRWQQGNVFSCSVMHEALHNHYTQKSLSLSPGK

SEQ ID NO: 10 - DNA, 681 bp, synthetic construct
  source 1..681: mol_type = other DNA
gacaaaactcacacatgcccaccgtgcccagcacctgaactcctggggggaccgtcagtcttcctcttccccccaaaacccaaggacaccctcatgatctcccggacccctgaggtcacatgcgtggtggtggacgtgagccacgaagaccctgaggtcaagttcaactggtacgtggacggcgtggaggtgcataatgccaagacaaagccgcgggaggagcagtacaacagcacgtaccgtgtggtcagcgtcctcaccgtcctgcaccaggactggctgaatggcaaggagtacaagtgcaaggtctccaacaaagccctcccagcccccatcgagaaaaccatctccaaagccaaagggcagccccgagaaccacaggtgtacaccctgcccccatcccgggatgagctgaccaagaaccaggtcagcctgacctgcctggtcaaaggcttctatcccagcgacatcgccgtggagtgggagagcaatgggcagccggagaacaactacaagaccacacctcccgtgctggactccgacggctccttcttcctctacagcaagctcaccgtggacaagagcaggtggcagcaggggaacgtcttctcatgctccgtgatgcatgaggctctgcacaaccactacacgcagaagagcctctccctgtctccgggtaaa